European Patent Specification EP 3 630 806 B1, published January 10, 2024. Title: Long-acting GIP Peptide Analogues. Applicant: University of Copenhagen. The sequence listing filed with the application follows.

SEQUENCE LISTING (148 sequences)

SEQ ID NO: 1 - protein, 25 aa, Artificial Sequence
  GIP analogues
  PEPTIDE (1)..(25): GIP analogues
FISDYSIAMDKIHQQDFVNWLLAQK

SEQ ID NO: 2 - protein, 28 aa, Artificial Sequence
  GIP analogues
  PEPTIDE (1)..(28): GIP analogues
EGTFISDYSIAMDKIHQQDFVNWLLAQK

SEQ ID NO: 3 - protein, 26 aa, Artificial Sequence
  GIP analogues
  PEPTIDE (7)..(7): is selected from the group consisting of S, K and Orn,
  PEPTIDE (8)..(8): is selected from the group consisting of I, K and Orn,
  PEPTIDE (9)..(9): is selected from the group consisting of A, K and Orn,
  PEPTIDE (10)..(10): is selected from the group consisting of M, K, L, S, Nle and Mox,
  PEPTIDE (11)..(11): is selected from the group consisting of D, E, A, K and Orn,
  PEPTIDE (12)..(12): is selected from the group consisting of K, R, A and E,
  PEPTIDE (14)..(14): is selected from the group consisting of H, A, R, K and Orn
  PEPTIDE (26)..(26): is selected from the group consisting of K, R, A and E
TFISDYXXXXXXIXQQDFVNWLLAQX

SEQ ID NO: 4 - protein, 28 aa, Artificial Sequence
  GIP analogues
  PEPTIDE (9)..(9): is selected from the group consisting of S, K and Orn,
  PEPTIDE (10)..(10): is selected from the group consisting of I, K and Orn,
  PEPTIDE (11)..(11): is selected from the group consisting of A, K and Orn,
  PEPTIDE (12)..(12): X14 is selected from the group consisting of M, K, L, S, Nle and Mox,
  PEPTIDE (13)..(13): is selected from the group consisting of D, E, A, K and Orn,
  PEPTIDE (14)..(14): is selected from the group consisting of K, R, A and E
  PEPTIDE (16)..(16): is selected from the group consisting of H, A, R, K and Orn
  PEPTIDE (28)..(28): is selected from the group consisting of K, R, A and E
EGTFISDYXXXXXXIXQQDFVNWLLAQX

SEQ ID NO: 5 - protein, 26 aa, Artificial Sequence
  GIP analogues
  PEPTIDE (1)..(26): GIP analogues
TFISDYSIAMDRIKQQDFVNWLLAQR

SEQ ID NO: 6 - protein, 26 aa, Artificial Sequence
  GIP analogues
  PEPTIDE (1)..(26): GIP analogues
TFISDYSIAMDRIHQQDFVNWLLAQR

SEQ ID NO: 7 - protein, 26 aa, Artificial Sequence
  GIP analogues
  PEPTIDE (1)..(26): GIP analogues
TFISDYSIAMDKIAQQDFVNWLLAQK

SEQ ID NO: 8 - protein, 26 aa, Artificial Sequence
  GIP analogues
  PEPTIDE (1)..(26): GIP analogues
TFISDYSIAMDKIKQQDFVNWLLAQK

SEQ ID NO: 9 - protein, 26 aa, Artificial Sequence
  GIP analogues
  PEPTIDE (1)..(1): GIP analogues
TFISDYSIAMEKIAQQDFVNWLLAQK

SEQ ID NO: 10 - protein, 26 aa, Artificial Sequence
  GIP analogues
  PEPTIDE (1)..(1): GIP analogues
TFISDYSIAMDAIAQQDFVNWLLAQK

SEQ ID NO: 11 - protein, 26 aa, Artificial Sequence
  GIP analogues
  PEPTIDE (1)..(1): GIP analogues
TFISDYSIAMEKIHQQDFVNWLLAQK

SEQ ID NO: 12 - protein, 26 aa, Artificial Sequence
  GIP analogues
  PEPTIDE (1)..(1): GIP analogues
TFISDYSIAMNKIHQQDFVNWLLAQK

SEQ ID NO: 13 - protein, 26 aa, Artificial Sequence
  GIP analogues
  PEPTIDE (1)..(1): GIP analogues
TFISDYSIAMDAIHQQDFVNWLLAQK

SEQ ID NO: 14 - protein, 26 aa, Artificial Sequence
  GIP analogues
  PEPTIDE (1)..(1): GIP analogues
TFISDYSIAMDHIHQQDFVNWLLAQK

SEQ ID NO: 15 - protein, 26 aa, Artificial Sequence
  GIP analogues
  PEPTIDE (1)..(1): GIP analogues
TFISDYSIAMDRIHQQDFVNWLLAQK

SEQ ID NO: 16 - protein, 26 aa, Artificial Sequence
  GIP analogues
  PEPTIDE (1)..(1): GIP analogues
TFISDYSIAMDKIFQQDFVNWLLAQK

SEQ ID NO: 17 - protein, 26 aa, Artificial Sequence
  GIP analogues
  PEPTIDE (1)..(1): GIP analogues
TFISDYSIAMDKIWQQDFVNWLLAQK

SEQ ID NO: 18 - protein, 26 aa, Artificial Sequence
  GIP analogues
  PEPTIDE (1)..(1): GIP analogues
TFISDYSIAMDKIHQQDFVNWLLAQR

SEQ ID NO: 19 - protein, 26 aa, Artificial Sequence
  GIP analogues
  PEPTIDE (1)..(1): GIP analogues
TFISDYSIAMDKIHQQDFVNWLLAQH

SEQ ID NO: 20 - protein, 26 aa, Artificial Sequence
  GIP analogues
  PEPTIDE (1)..(1): GIP analogues
KFISDYSIAMDKIHQQDFVNWLLAQK

SEQ ID NO: 21 - protein, 26 aa, Artificial Sequence
  GIP analogues
  PEPTIDE (1)..(1): GIP analogues
TKISDYSIAMDKIHQQDFVNWLLAQK

SEQ ID NO: 22 - protein, 26 aa, Artificial Sequence
  GIP analogues
  PEPTIDE (1)..(1): GIP analogues
TFKSDYSIAMDKIHQQDFVNWLLAQK

SEQ ID NO: 23 - protein, 26 aa, Artificial Sequence
  GIP analogues
  PEPTIDE (1)..(1): GIP analogues
TFIKDYSIAMDKIHQQDFVNWLLAQK

SEQ ID NO: 24 - protein, 26 aa, Artificial Sequence
  GIP analogues
  PEPTIDE (1)..(1): GIP analogues
TFISKYSIAMDKIHQQDFVNWLLAQK

SEQ ID NO: 25 - protein, 26 aa, Artificial Sequence
  GIP analogues
  PEPTIDE (1)..(1): GIP analogues
TFISDKSIAMDKIHQQDFVNWLLAQK

SEQ ID NO: 26 - protein, 26 aa, Artificial Sequence
  GIP analogues
  PEPTIDE (1)..(1): GIP analogues
TFISDYKIAMDKIHQQDFVNWLLAQK

SEQ ID NO: 27 - protein, 26 aa, Artificial Sequence
  GIP analogues
  PEPTIDE (1)..(1): GIP analogues
TFISDYSKAMDKIHQQDFVNWLLAQK

SEQ ID NO: 28 - protein, 26 aa, Artificial Sequence
  GIP analogues
  PEPTIDE (1)..(1): GIP analogues
TFISDYSIKMDKIHQQDFVNWLLAQK

SEQ ID NO: 29 - protein, 26 aa, Artificial Sequence
  GIP analogues
  PEPTIDE (1)..(1): GIP analogues
TFISDYSIAKDKIHQQDFVNWLLAQK

SEQ ID NO: 30 - protein, 26 aa, Artificial Sequence
  GIP analogues
  PEPTIDE (1)..(1): GIP analogues
TFISDYSIAMKKIHQQDFVNWLLAQK

SEQ ID NO: 31 - protein, 26 aa, Artificial Sequence
  GIP analogues
  PEPTIDE (1)..(1): GIP analogues
TFISDYSIAMDKKHQQDFVNWLLAQK

SEQ ID NO: 32 - protein, 26 aa, Artificial Sequence
  GIP analogues
  PEPTIDE (1)..(1): GIP analogues
TFISDYSIAMDKIHKQDFVNWLLAQK

SEQ ID NO: 33 - protein, 26 aa, Artificial Sequence
  GIP analogues
  PEPTIDE (1)..(1): GIP analogues
TFISDYSIAMDKIHQKDFVNWLLAQK

SEQ ID NO: 34 - protein, 26 aa, Artificial Sequence
  GIP analogues
  PEPTIDE (1)..(1): GIP analogues
TFISDYSIAMDKIHQQKFVNWLLAQK

SEQ ID NO: 35 - protein, 26 aa, Artificial Sequence
  GIP analogues
  PEPTIDE (1)..(1): GIP analogues
TFISDYSIAMDKIHQQDKVNWLLAQK

SEQ ID NO: 36 - protein, 26 aa, Artificial Sequence
  GIP analogues
  PEPTIDE (1)..(1): GIP analogues
TFISDYSIAMDKIHQQDFKNWLLAQK

SEQ ID NO: 37 - protein, 26 aa, Artificial Sequence
  GIP analogues
  PEPTIDE (1)..(1): GIP analogues
TFISDYSIAMDKIHQQDFVKWLLAQK

SEQ ID NO: 38 - protein, 26 aa, Artificial Sequence
  GIP analogues
  PEPTIDE (1)..(1): GIP analogues
TFISDYSIAMDKIHQQDFVNKLLAQK

SEQ ID NO: 39 - protein, 26 aa, Artificial Sequence
  GIP analogues
  PEPTIDE (1)..(1): GIP analogues
TFISDYSIAMDKIHQQDFVNWKLAQK

SEQ ID NO: 40 - protein, 26 aa, Artificial Sequence
  GIP analogues
  PEPTIDE (1)..(1): GIP analogues
TFISDYSIAMDKIHQQDFVNWLKAQK

SEQ ID NO: 41 - protein, 26 aa, Artificial Sequence
  GIP analogues
  PEPTIDE (1)..(11): GIP analogues
TFISDYSIAMDKIHQQDFVNWLLKQK

SEQ ID NO: 42 - protein, 26 aa, Artificial Sequence
  GIP analogues
  PEPTIDE (1)..(1): GIP analogues
TFISDYSIAMDKIHQQDFVNWLLAKK

SEQ ID NO: 43 - protein, 26 aa, Artificial Sequence
  GIP analogues
  PEPTIDE (1)..(11): GIP analogues
TFISDYKIAMDKIAQQDFVNWLLAQK

SEQ ID NO: 44 - protein, 26 aa, Artificial Sequence
  GIP analogues
  PEPTIDE (1)..(1): GIP analogues
TFISDYKIAMDKIRQQDFVNWLLAQK

SEQ ID NO: 45 - protein, 26 aa, Artificial Sequence
  GIP analogues
  PEPTIDE (1)..(1): GIP analogues
TFISDYKIAMEKIHQQDFVNWLLAQK

SEQ ID NO: 46 - protein, 26 aa, Artificial Sequence
  GIP analogues
  PEPTIDE (10)..(10): X = Nle
TFISDYKIAXDKIHQQDFVNWLLAQK

SEQ ID NO: 47 - protein, 26 aa, Artificial Sequence
  GIP analogues
  PEPTIDE (1)..(1): GIP analogues
TFISDYKIALDKIHQQDFVNWLLAQK

SEQ ID NO: 48 - protein, 26 aa, Artificial Sequence
  GIP analogues
  PEPTIDE (1)..(1): GIP analogues
TFISDYSKAMDKIAQQDFVNWLLAQK

SEQ ID NO: 49 - protein, 26 aa, Artificial Sequence
  GIP analogues
  PEPTIDE (1)..(1): GIP analogues
TFISDYSKAMDKIRQQDFVNWLLAQK

SEQ ID NO: 50 - protein, 26 aa, Artificial Sequence
  GIP analogues
  PEPTIDE (1)..(1): GIP analogues
TFISDYSKAMEKIHQQDFVNWLLAQK

SEQ ID NO: 51 - protein, 26 aa, Artificial Sequence
  GIP analogues
  PEPTIDE (10)..(10): X=Nle
TFISDYSKAXDKIHQQDFVNWLLAQK

SEQ ID NO: 52 - protein, 26 aa, Artificial Sequence
  GIP analogues
  PEPTIDE (1)..(1): GIP analogues
TFISDYSKALDKIHQQDFVNWLLAQK

SEQ ID NO: 53 - protein, 26 aa, Artificial Sequence
  GIP analogues
  PEPTIDE (1)..(1): GIP analogues
TFISDYSIKMDKIAQQDFVNWLLAQK

SEQ ID NO: 54 - protein, 26 aa, Artificial Sequence
  GIP analogues
  PEPTIDE (1)..(1): GIP analogues
TFISDYSIKMDKIRQQDFVNWLLAQK

SEQ ID NO: 55 - protein, 26 aa, Artificial Sequence
  GIP analogues
  PEPTIDE (1)..(1): GIP analogues
TFISDYSIKMEKIHQQDFVNWLLAQK

SEQ ID NO: 56 - protein, 26 aa, Artificial Sequence
  GIP analogues
  PEPTIDE (10)..(10): X=Nle
TFISDYSIKXDKIHQQDFVNWLLAQK

SEQ ID NO: 57 - protein, 26 aa, Artificial Sequence
  GIP analogues
  PEPTIDE (1)..(1): GIP analogues
TFISDYSIKLDKIHQQDFVNWLLAQK

SEQ ID NO: 58 - protein, 26 aa, Artificial Sequence
  GIP analogues
  PEPTIDE (1)..(1): GIP analogues
TFISDYSIAMEKIKQQDFVNWLLAQK

SEQ ID NO: 59 - protein, 26 aa, Artificial Sequence
  GIP analogues
  PEPTIDE (10)..(10): X=Nle
TFISDYSIAXDKIKQQDFVNWLLAQK

SEQ ID NO: 60 - protein, 28 aa, Artificial Sequence
  GIP analogues
  PEPTIDE (1)..(1): GIP analogues
TFISDYSIANLEDKIKQQDFVNWLLAQK

SEQ ID NO: 61 - protein, 26 aa, Artificial Sequence
  GIP analogues
  PEPTIDE (11)..(11): X=Orn
TFISDYSIAMXKIHQQDFVNWLLAQK

SEQ ID NO: 62 - protein, 26 aa, Artificial Sequence
  GIP analogues
  PEPTIDE (14)..(14): X=Orn
TFISDYSIAMDKIXQQDFVNWLLAQK

SEQ ID NO: 63 - protein, 26 aa, Artificial Sequence
  GIP analogues
  PEPTIDE (1)..(1): GIP analogues
TFISDYSIALDRIKQQDFVNWLLAQR

SEQ ID NO: 64 - protein, 26 aa, Artificial Sequence
  GIP analogues
  PEPTIDE (1)..(1): GIP analogues
KFISDYSIAMDRIHQQDFVNWLLAQR

SEQ ID NO: 65 - protein, 26 aa, Artificial Sequence
  GIP analogues
  PEPTIDE (1)..(1): GIP analogues
KFISDYSIAMDKIHQQDFVNWLLAQK

SEQ ID NO: 66 - protein, 26 aa, Artificial Sequence
  GIP analogues
  PEPTIDE (1)..(1): GIP analogues
TFISDYKIAMDRIHQQDFVNWLLAQR

SEQ ID NO: 67 - protein, 26 aa, Artificial Sequence
  GIP analogues
  PEPTIDE (1)..(1): GIP analogues
TFISDYKIALDRIHQQDFVNWLLAQR

SEQ ID NO: 68 - protein, 26 aa, Artificial Sequence
  GIP analogues
  PEPTIDE (1)..(1): GIP analogues
TFISDYSKAMDRIHQQDFVNWLLAQR

SEQ ID NO: 69 - protein, 26 aa, Artificial Sequence
  GIP analogues
  PEPTIDE (1)..(1): GIP analogues
TFISDYSKALDRIHQQDFVNWLLAQR

SEQ ID NO: 70 - protein, 26 aa, Artificial Sequence
  GIP analogues
  PEPTIDE (1)..(1): GIP analogues
TFISDYSIKMDRIHQQDFVNWLLAQR

SEQ ID NO: 71 - protein, 26 aa, Artificial Sequence
  GIP analogues
  PEPTIDE (1)..(1): GIP analogues
TFISDYSIKLDRIHQQDFVNWLLAQR

SEQ ID NO: 72 - protein, 28 aa, Artificial Sequence
  GIP analogues
  PEPTIDE (1)..(1): GIP analogues
EGTFISDYSIAMDRIKQQDFVNWLLAQR

SEQ ID NO: 73 - protein, 28 aa, Artificial Sequence
  GIP analogues
  PEPTIDE (1)..(1): GIP analogues
EGTFISDYSIAMDRIHQQDFVNWLLAQR

SEQ ID NO: 74 - protein, 28 aa, Artificial Sequence
  GIP analogues
  PEPTIDE (1)..(1): GIP analogues
EGTFISDYSIAMDKIAQQDFVNWLLAQK

SEQ ID NO: 75 - protein, 28 aa, Artificial Sequence
  GIP analogues
  PEPTIDE (1)..(1): GIP analogues
EGTFISDYSIAMDKIKQQDFVNWLLAQK

SEQ ID NO: 76 - protein, 28 aa, Artificial Sequence
  GIP analogues
  PEPTIDE (1)..(1): GIP analogues
EGTFISDYSIAMEKIAQQDFVNWLLAQK

SEQ ID NO: 77 - protein, 28 aa, Artificial Sequence
  GIP analogues
  PEPTIDE (1)..(1): GIP analogues
EGTFISDYSIAMDAIAQQDFVNWLLAQK

SEQ ID NO: 78 - protein, 28 aa, Artificial Sequence
  GIP analogues
  PEPTIDE (1)..(1): GIP analogues
EGTFISDYSIAMEKIHQQDFVNWLLAQK

SEQ ID NO: 79 - protein, 28 aa, Artificial Sequence
  GIP analogues
  PEPTIDE (1)..(1): GIP analogues
EGTFISDYSIAMNKIHQQDFVNWLLAQK

SEQ ID NO: 80 - protein, 28 aa, Artificial Sequence
  GIP analogues
  PEPTIDE (1)..(1): GIP analogues
EGTFISDYSIAMDAIHQQDFVNWLLAQK

SEQ ID NO: 81 - protein, 28 aa, Artificial Sequence
  GIP analogues
  PEPTIDE (1)..(1): GIP analogues
EGTFISDYSIAMDHIHQQDFVNWLLAQK

SEQ ID NO: 82 - protein, 28 aa, Artificial Sequence
  GIP analogues
  PEPTIDE (1)..(1): GIP analogues
EGTFISDYSIAMDRIHQQDFVNWLLAQK

SEQ ID NO: 83 - protein, 28 aa, Artificial Sequence
  GIP analogues
  PEPTIDE (1)..(1): GIP analogues
EGTFISDYSIAMDKIFQQDFVNWLLAQK

SEQ ID NO: 84 - protein, 28 aa, Artificial Sequence
  GIP analogues
  PEPTIDE (1)..(1): GIP analogues
EGTFISDYSIAMDKIWQQDFVNWLLAQK

SEQ ID NO: 85 - protein, 28 aa, Artificial Sequence
  GIP analogues
  PEPTIDE (1)..(1): GIP analogues
EGTFISDYSIAMDKIHQQDFVNWLLAQR

SEQ ID NO: 86 - protein, 28 aa, Artificial Sequence
  GIP analogues
  PEPTIDE (1)..(1): GIP analogues
EGTFISDYSIAMDKIHQQDFVNWLLAQH

SEQ ID NO: 87 - protein, 28 aa, Artificial Sequence
  GIP analogues
  PEPTIDE (1)..(1): GIP analogues
EKTFISDYSIAMDKIHQQDFVNWLLAQK

SEQ ID NO: 88 - protein, 28 aa, Artificial Sequence
  GIP analogues
  PEPTIDE (1)..(1): GIP analogues
EGKFISDYSIAMDKIHQQDFVNWLLAQK

SEQ ID NO: 89 - protein, 28 aa, Artificial Sequence
  GIP analogues
  PEPTIDE (1)..(1): GIP analogues
EGTKISDYSIAMDKIHQQDFVNWLLAQK

SEQ ID NO: 90 - protein, 28 aa, Artificial Sequence
  GIP analogues
  PEPTIDE (1)..(1): GIP analogues
EGTFKSDYSIAMDKIHQQDFVNWLLAQK

SEQ ID NO: 91 - protein, 28 aa, Artificial Sequence
  GIP analogues
  PEPTIDE (1)..(1): GIP analogues
EGTFIKDYSIAMDKIHQQDFVNWLLAQK

SEQ ID NO: 92 - protein, 28 aa, Artificial Sequence
  GIP analogues
  PEPTIDE (1)..(1): GIP analogues
EGTFISKYSIAMDKIHQQDFVNWLLAQK

SEQ ID NO: 93 - protein, 28 aa, Artificial Sequence
  GIP analogues
  PEPTIDE (1)..(1): GIP analogues
EGTFISDKSIAMDKIHQQDFVNWLLAQK

SEQ ID NO: 94 - protein, 28 aa, Artificial Sequence
  GIP analogues
  PEPTIDE (1)..(1): GIP analogues
EGTFISDYKIAMDKIHQQDFVNWLLAQK

SEQ ID NO: 95 - protein, 28 aa, Artificial Sequence
  GIP analogues
  PEPTIDE (1)..(1): GIP analogues
EGTFISDYSKAMDKIHQQDFVNWLLAQK

SEQ ID NO: 96 - protein, 28 aa, Artificial Sequence
  GIP analogues
  PEPTIDE (1)..(1): GIP analogues
EGTFISDYSIKMDKIHQQDFVNWLLAQK

SEQ ID NO: 97 - protein, 28 aa, Artificial Sequence
  GIP analogues
  PEPTIDE (1)..(1): GIP analogues
EGTFISDYSIAKDKIHQQDFVNWLLAQK

SEQ ID NO: 98 - protein, 28 aa, Artificial Sequence
  GIP analogues
  PEPTIDE (1)..(1): GIP analogues
EGTFISDYSIAMKKIHQQDFVNWLLAQK

SEQ ID NO: 99 - protein, 28 aa, Artificial Sequence
  GIP analogues
  PEPTIDE (1)..(1): GIP analogues
EGTFISDYSIAMDKKHQQDFVNWLLAQK

SEQ ID NO: 100 - protein, 28 aa, Artificial Sequence
  GIP analogues
  PEPTIDE (1)..(1): GIP analogues
EGTFISDYSIAMDKIHKQDFVNWLLAQK

SEQ ID NO: 101 - protein, 28 aa, Artificial Sequence
  GIP analogues
  PEPTIDE (1)..(1): GIP analogues
EGTFISDYSIAMDKIHQKDFVNWLLAQK

SEQ ID NO: 102 - protein, 28 aa, Artificial Sequence
  GIP analogues
  PEPTIDE (1)..(1): GIP analogues
EGTFISDYSIAMDKIHQQKFVNWLLAQK

SEQ ID NO: 103 - protein, 28 aa, Artificial Sequence
  GIP analogues
  PEPTIDE (1)..(1): GIP analogues
EGTFISDYSIAMDKIHQQDKVNWLLAQK

SEQ ID NO: 104 - protein, 28 aa, Artificial Sequence
  GIP analogues
  PEPTIDE (1)..(1): GIP analogues
EGTFISDYSIAMDKIHQQDFKNWLLAQK

SEQ ID NO: 105 - protein, 28 aa, Artificial Sequence
  GIP analogues
  PEPTIDE (1)..(1): GIP analogues
EGTFISDYSIAMDKIHQQDFVKWLLAQK

SEQ ID NO: 106 - protein, 28 aa, Artificial Sequence
  GIP analogues
  PEPTIDE (1)..(1): GIP analogues
EGTFISDYSIAMDKIHQQDFVNKLLAQK

SEQ ID NO: 107 - protein, 28 aa, Artificial Sequence
  GIP analogues
  PEPTIDE (1)..(1): GIP analogues
EGTFISDYSIAMDKIHQQDFVNWKLAQK

SEQ ID NO: 108 - protein, 28 aa, Artificial Sequence
  GIP analogues
  PEPTIDE (1)..(1): GIP analogues
EGTFISDYSIAMDKIHQQDFVNWLKAQK

SEQ ID NO: 109 - protein, 28 aa, Artificial Sequence
  GIP analogues
  PEPTIDE (1)..(1): GIP analogues
EGTFISDYSIAMDKIHQQDFVNWLLKQK

SEQ ID NO: 110 - protein, 28 aa, Artificial Sequence
  GIP analogues
  PEPTIDE (1)..(1): GIP analogues
EGTFISDYSIAMDKIHQQDFVNWLLAKK

SEQ ID NO: 111 - protein, 28 aa, Artificial Sequence
  GIP analogues
  PEPTIDE (1)..(1): GIP analogues
EGTFISDYKIAMDKIAQQDFVNWLLAQK

SEQ ID NO: 112 - protein, 28 aa, Artificial Sequence
  GIP analogues
  PEPTIDE (1)..(1): GIP analogues
EGTFISDYKIAMDKIRQQDFVNWLLAQK

SEQ ID NO: 113 - protein, 28 aa, Artificial Sequence
  GIP analogues
  PEPTIDE (1)..(1): GIP analogues
EGTFISDYKIAMEKIHQQDFVNWLLAQK

SEQ ID NO: 114 - protein, 28 aa, Artificial Sequence
  GIP analogues
  PEPTIDE (12)..(12): X=Nle
EGTFISDYKIAXDKIHQQDFVNWLLAQK

SEQ ID NO: 115 - protein, 28 aa, Artificial Sequence
  GIP analogues
  PEPTIDE (1)..(1): GIP analogues
EGTFISDYKIALDKIHQQDFVNWLLAQK

SEQ ID NO: 116 - protein, 28 aa, Artificial Sequence
  GIP analogues
  PEPTIDE (1)..(1): GIP analogues
EGTFISDYSKAMDKIAQQDFVNWLLAQK

SEQ ID NO: 117 - protein, 28 aa, Artificial Sequence
  GIP analogues
  PEPTIDE (1)..(1): GIP analogues
EGTFISDYSKAMDKIRQQDFVNWLLAQK

SEQ ID NO: 118 - protein, 28 aa, Artificial Sequence
  GIP analogues
  PEPTIDE (1)..(1): GIP analogues
EGTFISDYSKAMEKIHQQDFVNWLLAQK

SEQ ID NO: 119 - protein, 28 aa, Artificial Sequence
  GIP analogues
  PEPTIDE (12)..(12): X=Nle
EGTFISDYSKAXDKIHQQDFVNWLLAQK

SEQ ID NO: 120 - protein, 28 aa, Artificial Sequence
  GIP analogues
  PEPTIDE (1)..(1): GIP analogues
EGTFISDYSKALDKIHQQDFVNWLLAQK

SEQ ID NO: 121 - protein, 28 aa, Artificial Sequence
  GIP analogues
  PEPTIDE (1)..(1): GIP analogues
EGTFISDYSIKMDKIAQQDFVNWLLAQK

SEQ ID NO: 122 - protein, 28 aa, Artificial Sequence
  GIP analogues
  PEPTIDE (1)..(1): GIP analogues
EGTFISDYSIKMDKIRQQDFVNWLLAQK

SEQ ID NO: 123 - protein, 28 aa, Artificial Sequence
  GIP analogues
  PEPTIDE (1)..(1): GIP analogues
EGTFISDYSIKMEKIHQQDFVNWLLAQK

SEQ ID NO: 124 - protein, 28 aa, Artificial Sequence
  GIP analogues
  PEPTIDE (12)..(12): X=Nle
EGTFISDYSIKXDKIHQQDFVNWLLAQK

SEQ ID NO: 125 - protein, 28 aa, Artificial Sequence
  GIP analogues
  PEPTIDE (1)..(1): GIP analogues
EGTFISDYSIKLDKIHQQDFVNWLLAQK

SEQ ID NO: 126 - protein, 28 aa, Artificial Sequence
  GIP analogues
  PEPTIDE (1)..(1): GIP analogues
EGTFISDYSIAMEKIKQQDFVNWLLAQK

SEQ ID NO: 127 - protein, 28 aa, Artificial Sequence
  GIP analogues
  PEPTIDE (12)..(12): X=Nle
EGTFISDYSIAXDKIKQQDFVNWLLAQK

SEQ ID NO: 128 - protein, 28 aa, Artificial Sequence
  GIP analogues
  PEPTIDE (1)..(1): GIP analogues
EGTFISDYSIALDKIKQQDFVNWLLAQK

SEQ ID NO: 129 - protein, 28 aa, Artificial Sequence
  GIP analogues
  PEPTIDE (1)..(1): GIP analogues
EGKFISDYSIAMDRIHQQDFVNWLLAQR

SEQ ID NO: 130 - protein, 28 aa, Artificial Sequence
  GIP analogues
  PEPTIDE (13)..(13): X=Orn
EGTFISDYSIAMXKIHQQDFVNWLLAQK

SEQ ID NO: 131 - protein, 28 aa, Artificial Sequence
  GIP analogues
  PEPTIDE (16)..(16): X=Orn
EGTFISDYSIAMDKIXQQDFVNWLLAQK

SEQ ID NO: 132 - protein, 28 aa, Artificial Sequence
  GIP analogues
  PEPTIDE (1)..(1): GIP analogues
EGTFISDYSIALDRIKQQDFVNWLLAQR

SEQ ID NO: 133 - protein, 26 aa, Artificial Sequence
  GIP analogues
  PEPTIDE (7)..(7): X=Orn
TFISDYXIAMDKIHQQDFVNWLLAQK

SEQ ID NO: 134 - protein, 28 aa, Artificial Sequence
  GIP analogues
  PEPTIDE (9)..(9): X=Orn
EGTFISDYXIAMDKIHQQDFVNWLLAQK

SEQ ID NO: 135 - protein, 26 aa, Artificial Sequence
  GIP analogues
  PEPTIDE (8)..(8): X=Orn
TFISDYSXAMDKIHQQDFVNWLLAQK

SEQ ID NO: 136 - protein, 28 aa, Artificial Sequence
  GIP analogues
  PEPTIDE (10)..(10): X=Orn
EGTFISDYSXAMDKIHQQDFVNWLLAQK

SEQ ID NO: 137 - protein, 26 aa, Artificial Sequence
  GIP analogues
  PEPTIDE (9)..(9): X=Orn
TFISDYSIXMDKIHQQDFVNWLLAQK

SEQ ID NO: 138 - protein, 28 aa, Artificial Sequence
  GIP analogues
  PEPTIDE (11)..(11): X=Orn
EGTFISDYSIXMDKIHQQDFVNWLLAQK

SEQ ID NO: 139 - protein, 26 aa, Artificial Sequence
  GIP analogues
  PEPTIDE (17)..(17): X=Orn
TFISDYSIAMDKIHQQXFVNWLLAQK

SEQ ID NO: 140 - protein, 28 aa, Artificial Sequence
  GIP analogues
  PEPTIDE (19)..(19): X=Orn
EGTFISDYSIAMDKIHQQXFVNWLLAQK

SEQ ID NO: 141 - protein, 28 aa, Artificial Sequence
  GIP analogues
  PEPTIDE (3)..(3): X=Orn
EGXFISDYSIAMDKIHQQKFVNWLLAQK

SEQ ID NO: 142 - protein, 28 aa, Artificial Sequence
  GIP analogues
  PEPTIDE (13)..(13): X=Orn
EGTFISDYSIAMXKIHQQKFVNWLLAQK

SEQ ID NO: 143 - protein, 28 aa, Artificial Sequence
  GIP analogues
  PEPTIDE (18)..(18): X=Orn
EGTFISDYSIAMDKIHQXKFVNWLLAQK

SEQ ID NO: 144 - protein, 28 aa, Artificial Sequence
  GIP analogues
  PEPTIDE (1)..(1): GIP analogues
EGWFISDYSIAMEKIAQQDFVNWLLAQK

SEQ ID NO: 145 - protein, 26 aa, Artificial Sequence
  GIP analogues
  PEPTIDE (1)..(1): GIP analogues
TFISDYSIAMDRIHQQKFVNWLLAQR

SEQ ID NO: 146 - protein, 28 aa, Artificial Sequence
  GIP analogues
  PEPTIDE (1)..(1): GIP analogues
EGTFISDYSIAMDKIKQQDFVNWLLAQR

SEQ ID NO: 147 - protein, 25 aa, Artificial Sequence
  hGIP6-30
  PEPTIDE (1)..(1): hGIP6-30
FISDYSIAMDKIHQQDFVNWLLAQK

SEQ ID NO: 148 - protein, 27 aa, Artificial Sequence
  hGIP4-30
  PEPTIDE (1)..(1): hGIP4-30
GTFISDYSIAMDKIHQQDFVNWLLAQK